European Patent Application EP 4 365 311 A2, published May 8, 2024. Title: METHODS OF DETECTING LENTIVIRUS. Applicant: ST VINCENT'S HOSPITAL SYDNEY LIMITED. Application EP. The sequence listing filed with the application follows.

SEQUENCE LISTING (55 sequences)

SEQ ID NO: 1 - DNA, 95 bp, Human immunodeficiency virus type 1
  source 1..95: mol_type = other DNA
gtctctctggttagaccagatctgagcctgggagctctctggctaactagggaacccactgcttaagcctcaataaagcttgccttgagtgcttc

SEQ ID NO: 2 - DNA, 124 bp, Human immunodeficiency virus type 2
  source 1..124: mol_type = other DNA
ttgagccctgggaggttctctccagcactagcaggtagagcctgggtgttccctgctagactctcaccagcacttggccggtgctgggcagacggccccacgcttgcttgcttaaaaacctcct

SEQ ID NO: 3 - DNA, 17 bp, Human immunodeficiency virus type 1
  source 1..17: mol_type = other DNA
taagcagtgggttccct

SEQ ID NO: 4 - DNA, 17 bp, synthetic construct
  misc_feature 1..17: note = Sequence of the HIV-1 R region probe oligo
  source 1..17: mol_type = other DNA
agggaacccactgctta

SEQ ID NO: 5 - DNA, 17 bp, synthetic construct
  misc_feature 1..17: note = Sequence of the HIV-1 R region probe oligo with reporter and quencher
  misc_feature 1: note = Adenine is attached with X wherein X is a reporter molecule
  misc_feature 17: note = Adenine is attached with Z wherein Z is a quencher molecule.
  source 1..17: mol_type = other DNA
agggaacccactgctta

SEQ ID NO: 6 - DNA, 17 bp, synthetic construct
  misc_feature 1..17: note = Sequence of the HIV-1 R region probe oligo with locked nucleic acids
  misc_feature 1: note = Adenine is attached with FAM (carboxyfluorescein)
  misc_feature 17: note = Adenine is attached with BHQ-1
  source 1..17: mol_type = other DNA
  misc_feature 3: note = backbone sugar is a locked nucleic acid (LNA)
  misc_feature 5: note = backbone sugar is a locked nucleic acid (LNA)
  misc_feature 7: note = backbone sugar is a locked nucleic acid (LNA)
  misc_feature 11: note = backbone sugar is a locked nucleic acid (LNA)
  misc_feature 13: note = backbone sugar is a locked nucleic acid (LNA)
agggaacccactgctta

SEQ ID NO: 7 - DNA, 18 bp, synthetic construct
  source 1..18: mol_type = other DNA
gagcctgggagctctctg

SEQ ID NO: 8 - DNA, 18 bp, Human immunodeficiency virus type 1
  source 1..18: mol_type = other DNA
cagagagctcccaggctc

SEQ ID NO: 9 - DNA, 24 bp, synthetic construct
  misc_feature 1..24: note = HIV-1 reverse R region primer
  source 1..24: mol_type = other DNA
actcaaggcaagctttattgaggc

SEQ ID NO: 10 - DNA, 24 bp, Human immunodeficiency virus type 1
  source 1..24: mol_type = other DNA
gcctcaataaagcttgccttgagt

SEQ ID NO: 11 - DNA, 25 bp, Human immunodeficiency virus type 2
  source 1..25: mol_type = other DNA
gcctgggtgttccctgctagactct

SEQ ID NO: 12 - DNA, 25 bp, synthetic construct
  misc_feature 1..25: note = Sequence of the HIV-2 R region probe oligo
  source 1..25: mol_type = other DNA
agagtctagcagggaacacccaggc

SEQ ID NO: 13 - DNA, 25 bp, synthetic construct
  misc_feature 1..25: note = Sequence of the HIV-2 R region probe oligo with reporter and quencher
  misc_feature 1: note = Adenine is attached with X wherein X is a reporter molecule
  misc_feature 25: note = Cytosine is attached with Z wherein Z is a quencher molecule
  source 1..25: mol_type = other DNA
agagtctagcagggaacacccaggc

SEQ ID NO: 14 - DNA, 18 bp, synthetic construct
  misc_feature 1..18: note = HIV-2 forward R region primer
  source 1..18: mol_type = other DNA
gagccctgagaggttctc

SEQ ID NO: 15 - DNA, 18 bp, Human immunodeficiency virus type 2
  source 1..18: mol_type = other DNA
gagaacctcccagggctc

SEQ ID NO: 16 - DNA, 23 bp, synthetic construct
  misc_feature 1..23: note = HIV-2 reverse R region primer
  source 1..23: mol_type = other DNA
ggtctttaagcaagcaagcgtgg

SEQ ID NO: 17 - DNA, 27 bp, synthetic construct
  misc_feature 1..27: note = GAPDH probe oligo
  misc_feature 1: note = Adenine is attached with FAM (carboxyfluorescein)
  misc_feature 27: note = Thymine is attached with quencher molecule BHQ-1
  source 1..27: mol_type = other DNA
aaggtcggagtcaacggatttggtcgt

SEQ ID NO: 18 - DNA, 23 bp, synthetic construct
  misc_feature 1..23: note = GAPDH forward primer
  source 1..23: mol_type = other DNA
ggcaacaatatccactttaccag

SEQ ID NO: 19 - DNA, 20 bp, synthetic construct
  misc_feature 1..20: note = GAPDH reverse primer
  source 1..20: mol_type = other DNA
tcgacagtcagccgcatctt

SEQ ID NO: 20 - DNA, 25 bp, synthetic construct
  misc_feature 1..25: note = B-actin probe oligo
  misc_feature 1: note = Adenine is attached with FAM (carboxyfluorescein)
  misc_feature 25: note = Guanine is attached with quencher molecule BHQ-1
  source 1..25: mol_type = other DNA
atgccctcccccatgccatcctgcg

SEQ ID NO: 21 - DNA, 25 bp, synthetic construct
  misc_feature 1..25: note = B-actin forward primer
  source 1..25: mol_type = other DNA
tcacccacactgtgcccatctacga

SEQ ID NO: 22 - DNA, 25 bp, synthetic construct
  misc_feature 1..25: note = B-actin reverse primer
  source 1..25: mol_type = other DNA
cagcggaaccgctcattgccaatgg

SEQ ID NO: 23 - DNA, 24 bp, synthetic construct
  misc_feature 1..24: note = 3' LTR forward primer
  source 1..24: mol_type = other DNA
ccaaagaagacaagatatccttga

SEQ ID NO: 24 - DNA, 18 bp, synthetic construct
  misc_feature 1..18: note = 3' LTR reverse primer
  source 1..18: mol_type = other DNA
ttgaggcttaagcagtgg

SEQ ID NO: 25 - DNA, 29 bp, synthetic construct
  misc_feature 1..29: note = 3' LTR probe oligo
  misc_feature 1: note = Thymine is attached with FAM (carboxyfluorescein)
  misc_feature 29: note = Cytosine is attached with quencher molecule BHQ-1
  source 1..29: mol_type = other DNA
ttagaccagatctgagcctgggagctctc

SEQ ID NO: 26 - DNA, 30 bp, synthetic construct
  misc_feature 1..30: note = gag forward primer
  source 1..30: mol_type = other DNA
agtggggggacatcaagcagccatgcaaat

SEQ ID NO: 27 - DNA, 28 bp, synthetic construct
  misc_feature 1..28: note = gag reverse primer
  source 1..28: mol_type = other DNA
tactagtagttcctgctatgtcacttcc

SEQ ID NO: 28 - DNA, 17 bp, synthetic construct
  misc_feature 1..17: note = gag probe oligo
  misc_feature 1: note = Adenine is attached with FAM (carboxyfluorescein)
  misc_feature 17: note = Cytosine is attached with quencher molecule BHQ-1
  source 1..17: mol_type = other DNA
  misc_feature 3: note = backbone sugar is a locked nucleic acid (LNA)
  misc_feature 4: note = backbone sugar is a locked nucleic acid (LNA)
  misc_feature 7: note = backbone sugar is a locked nucleic acid (LNA)
  misc_feature 13: note = backbone sugar is a locked nucleic acid (LNA)
  misc_feature 16: note = backbone sugar is a locked nucleic acid (LNA)
atcaatgaggaagctgc

SEQ ID NO: 29 - DNA, 18 bp, synthetic construct
  misc_feature 1..18: note = HIV-1 forward R region primer (HIV-1 For 2)
  misc_feature 6: note = T or C
  misc_feature 15: note = T or C
  source 1..18: mol_type = other DNA
gagccngggagctcnctg

SEQ ID NO: 30 - DNA, 22 bp, synthetic construct
  misc_feature 1..22: note = HIV-1 reverse R region primer (HIV-1 Rev 2)
  source 1..22: mol_type = other DNA
actcaaggcaagctttattgag

SEQ ID NO: 31 - DNA, 18 bp, synthetic construct
  misc_feature 1..18: note = HIV-2 forward R region primer (HIV-2 For 1)
  misc_feature 9: note = G or A
  source 1..18: mol_type = other DNA
gagccctgngaggttctc

SEQ ID NO: 32 - DNA, 23 bp, synthetic construct
  misc_feature 1..23: note = HIV-2 reverse R region primer (HIV-2 Rev 1)
  misc_feature 4: note = T or C
  source 1..23: mol_type = other DNA
ggtntttaagcaagcaagcgtgg

SEQ ID NO: 33 - DNA, 18 bp, synthetic construct
  misc_feature 1..18: note = HIV-2 forward R region primer (HIV-2 For 2)
  misc_feature 9: note = G or A
  source 1..18: mol_type = other DNA
gagccctgngaggttctc

SEQ ID NO: 34 - DNA, 18 bp, synthetic construct
  misc_feature 1..18: note = HIV-2 reverse R region primer (HIV-2 Rev 2)
  source 1..18: mol_type = other DNA
agggaacacccaggctct

SEQ ID NO: 35 - DNA, 19 bp, synthetic construct
  misc_feature 1..19: note = HIV-2 forward R region primer (HIV 2 For 3)
  source 1..19: mol_type = other DNA
ttgagccctgggaggttct

SEQ ID NO: 36 - DNA, 18 bp, synthetic construct
  misc_feature 1..18: note = HIV-2 reverse R region primer (HIV-2 Rev 3)
  source 1..18: mol_type = other DNA
ggaacacccaggctctac

SEQ ID NO: 37 - DNA, 14 bp, synthetic construct
  misc_feature 1..14: note = Sequence of the HIV-2 R region probe oligo (HIV-2 Pro 2)
  source 1..14: mol_type = other DNA
ctgctagtgctgga

SEQ ID NO: 38 - DNA, 14 bp, synthetic construct
  misc_feature 1..14: note = Sequence of the HIV-2 R region probe oligo (HIV-2 Pro 2) with reporter and quencher
  misc_feature 1: note = Cytosine is attached with X wherein X is a reporter molecule
  misc_feature 14: note = Adenine is attached with Z wherein Z is a quencher molecule
  source 1..14: mol_type = other DNA
ctgctagtgctgga

SEQ ID NO: 39 - DNA, 14 bp, synthetic construct
  misc_feature 1..14: note = Sequence of the HIV-2 R region probe oligo (HIV-2 Pro 2) with FAM and BHQ-1
  misc_feature 1: note = Cytosine is attached with FAM (carboxyfluorescein)
  misc_feature 14: note = Adenine is attached with quencher molecule BHQ-1
  source 1..14: mol_type = other DNA
ctgctagtgctgga

SEQ ID NO: 40 - DNA, 14 bp, synthetic construct
  misc_feature 1..14: note = Sequence of the HIV-2 R region probe oligo (HIV-2 Pro 2) with locked nucleic acids, FAM and BHQ-1
  misc_feature 1: note = Cytosine is attached with FAM (carboxyfluorescein)
  misc_feature 14: note = Adenine is attached with quencher molecule BHQ-1
  source 1..14: mol_type = other DNA
  misc_feature 2: note = backbone sugar is a locked nucleic acid (LNA)
  misc_feature 4: note = backbone sugar is a locked nucleic acid (LNA)
  misc_feature 6: note = backbone sugar is a locked nucleic acid (LNA)
  misc_feature 8: note = backbone sugar is a locked nucleic acid (LNA)
  misc_feature 9: note = backbone sugar is a locked nucleic acid (LNA)
  misc_feature 13: note = backbone sugar is a locked nucleic acid (LNA)
ctgctagtgctgga

SEQ ID NO: 41 - DNA, 14 bp, synthetic construct
  misc_feature 1..14: note = Sequence of the HIV-2 R region probe oligo (HIV-2 Pro 3)
  source 1..14: mol_type = other DNA
tccagcactagcag

SEQ ID NO: 42 - DNA, 14 bp, synthetic construct
  misc_feature 1..14: note = Sequence of the HIV-2 R region probe oligo (HIV-2 Pro 3) with reporter and quencher
  misc_feature 1: note = Thymine is attached with X wherein X is a reporter molecule
  misc_feature 14: note = Guanine is attached with Z wherein Z is a quencher molecule
  source 1..14: mol_type = other DNA
tccagcactagcag

SEQ ID NO: 43 - DNA, 14 bp, synthetic construct
  misc_feature 1..14: note = Sequence of the HIV-2 R region probe oligo (HIV-2 Pro 3) with FAM and BHQ-1
  misc_feature 1: note = Thymine is attached with FAM (carboxyfluorescein)
  misc_feature 14: note = Guanine is attached with quencher molecule BHQ-1
  source 1..14: mol_type = other DNA
tccagcactagcag

SEQ ID NO: 44 - DNA, 14 bp, synthetic construct
  misc_feature 1..14: note = Sequence of the HIV-2 R region probe oligo (HIV-2 Pro 3) with locked nucleic acids, FAM and BHQ-1
  misc_feature 1: note = Thymine is attached with FAM (carboxyfluorescein)
  misc_feature 14: note = Guanine is attached with quencher molecule BHQ-1
  source 1..14: mol_type = other DNA
  misc_feature 2: note = backbone sugar is a locked nucleic acid (LNA)
  misc_feature 4: note = backbone sugar is a locked nucleic acid (LNA)
  misc_feature 6: note = backbone sugar is a locked nucleic acid (LNA)
  misc_feature 8: note = backbone sugar is a locked nucleic acid (LNA)
  misc_feature 10: note = backbone sugar is a locked nucleic acid (LNA)
  misc_feature 12: note = backbone sugar is a locked nucleic acid (LNA)
tccagcactagcag

SEQ ID NO: 45 - DNA, 30 bp, synthetic construct
  misc_feature 1..15: note = up to 5 T nucleotides may be added to the 5' terminus, or up to 10 T nucleotides may be deleted from the 5' terminus
  source 1..30: mol_type = other DNA
tttttttttttttttggaacccactgctta

SEQ ID NO: 46 - DNA, 15 bp, synthetic construct
  misc_feature 1..15: note = Sequence of the HIV-1 R region probe oligo (HIV-1 Pro 2) with reporter and quencher
  misc_feature 1: note = Guanine is attached with X wherein X is a reporter molecule
  misc_feature 15: note = Adenine is attached with Z wherein Z is a quencher molecule
  source 1..15: mol_type = other DNA
ggaacccactgctta

SEQ ID NO: 47 - DNA, 15 bp, synthetic construct
  misc_feature 1..15: note = Sequence of the HIV-1 R region probe oligo (HIV-1 Pro 3)
  source 1..15: mol_type = other DNA
agggaacccactgct

SEQ ID NO: 48 - DNA, 15 bp, synthetic construct
  misc_feature 1..15: note = Sequence of the HIV-1 R region probe oligo (HIV-1 Pro 3) with reporter and quencher
  misc_feature 1: note = Adenine is attached with X wherein X is a reporter molecule
  misc_feature 15: note = Thymine is attached with Z wherein Z is a quencher molecule
  source 1..15: mol_type = other DNA
agggaacccactgct

SEQ ID NO: 49 - DNA, 30 bp, synthetic construct
  misc_feature 1..17: note = Sequence of the HIV-2 R region probe oligo (HIV-2 Pro 4)
  misc_feature 1..15: note = Up to 5 T nucleotides may be added to the 5' terminus or up to 10 T nucleotides may be removed from the 5' terminus
  source 1..30: mol_type = other DNA
tttttttttttttttccagcactagcaggt

SEQ ID NO: 50 - DNA, 16 bp, synthetic construct
  misc_feature 1..16: note = Sequence of the HIV-2 R region probe oligo (HIV-2 Pro 4) with reporter and quencher
  misc_feature 1: note = Thymine is attached with X wherein X is a reporter molecule
  misc_feature 16: note = Thymine is attached with Z wherein Z is a quencher molecule
  source 1..16: mol_type = other DNA
tccagcactagcaggt

SEQ ID NO: 51 - DNA, 15 bp, synthetic construct
  misc_feature 1..15: note = Sequence of the HIV-2 R region probe oligo (HIV-2 Pro 5)
  source 1..15: mol_type = other DNA
ctccagcactagcag

SEQ ID NO: 52 - DNA, 15 bp, synthetic construct
  misc_feature 1..15: note = Sequence of the HIV-2 R region probe oligo (HIV-2 Pro 5) with reporter and quencher
  misc_feature 1: note = Cytosine is attached with X wherein X is a reporter molecule
  misc_feature 15: note = Guanine is attached with Z wherein Z is a quencher molecule
  source 1..15: mol_type = other DNA
ctccagcactagcag

SEQ ID NO: 53 - DNA, 15 bp, synthetic construct
  misc_feature 1..15: note = Sequence of the HIV-2 R region probe oligo (HIV-2 Pro-5) with locked nucleic acids
  source 1..15: mol_type = other DNA
  misc_feature 2: note = backbone sugar is a locked nucleic acid (LNA)
  misc_feature 5: note = backbone sugar is a locked nucleic acid (LNA)
  misc_feature 6: note = backbone sugar is a locked nucleic acid (LNA)
  misc_feature 8: note = backbone sugar is a locked nucleic acid (LNA)
  misc_feature 11: note = backbone sugar is a locked nucleic acid (LNA)
  misc_feature 13: note = backbone sugar is a locked nucleic acid (LNA)
ctccagcactagcag

SEQ ID NO: 54 - DNA, 35 bp, synthetic construct
  source 1..35: mol_type = other DNA
  misc_feature 1..20: note = up to 15 T nucleotides may be removed from the 5' terminus
ttttttttttttttttttttggaacccactgctta

SEQ ID NO: 55 - DNA, 35 bp, synthetic construct
  source 1..35: mol_type = other DNA
  misc_feature 1..20: note = up to 15 T nucleotides may be removed from the 5' terminus
ttttttttttttttttttttccagcagtagcaggt